European Patent Specification EP 3 754 335 B1, published November 22, 2023. Title: Target substance detection method, target substance detection kit, and target substance detection system. Applicant: ARKRAY, Inc. The sequence listing filed with the application follows.

SEQUENCE LISTING (3 sequences)

SEQ ID NO: 1 - DNA, 24 bp, Artificial Sequence
  Binding part
tttttttttttttttttttttttt

SEQ ID NO: 2 - RNA, 99 nt, Artificial Sequence
  Nucleic acid aptamer probe 1.
gggagaauuccgaccagaagaauaguagaaugagcucugucggacccagccuuuccucucuccuuccucuucuuuaaaaaaaaaaaaaaaaaaaaaaaa

SEQ ID NO: 3 - RNA, 61 nt, Artificial Sequence
  Nucleic acid aptamer probe 2.
ggguuagcagucggcaugcgguacagacagacccuuuaaaaaaaaaaaaaaaaaaaaaaaa